European Patent Specification EP 3 428 183 B1, published March 20, 2024. Title: SULFATION OF WNT PATHWAY PROTEINS. Applicant: RABBANI, JOSHUA DONEGAN, JAMES J. LI, XIAOFENG. Application 13/170,634. The sequence listing filed with the application follows.

SEQUENCE LISTING (31 sequences)

SEQ ID NO: 1 - protein, 12 aa, Homo sapiens
DNYQPYPCAEDE

SEQ ID NO: 2 - protein, 12 aa, Homo sapiens
LGEYPEPPPELE

SEQ ID NO: 3 - protein, 8 aa, Homo sapiens
YVTDGPCR

SEQ ID NO: 4 - protein, 10 aa, Homo sapiens
ANQAELENAY

SEQ ID NO: 5 - protein, 16 aa, Homo sapiens
ELGEYPEPPPELENNK

SEQ ID NO: 6 - protein, 16 aa, Mus musculus
GLGEYPEPPPENNQTM

SEQ ID NO: 7 - protein, 16 aa, Rattus norvegicus
GLREYPEPPQELENNQ

SEQ ID NO: 8 - protein, 11 aa, Homo sapiens
KANQAELENAY

SEQ ID NO: 9 - protein, 13 aa, Artificial Sequence
  Description of Artificial Sequence: Synthetic peptide
ELGEYPEPPPELE

SEQ ID NO: 10 - protein, 11 aa, Artificial Sequence
  Description of Artificial Sequence: Synthetic peptide
KANQAELENAY

SEQ ID NO: 11 - DNA, 20 bp, Artificial Sequence
  Description of Artificial Sequence: Synthetic primer
caggggtggcaggcgttcaa

SEQ ID NO: 12 - DNA, 20 bp, Artificial Sequence
  Description of Artificial Sequence: Synthetic primer
gtaggcgttctccagctcgg

SEQ ID NO: 13 - protein, 9 aa, Homo sapiens
IIYHMDEEE

SEQ ID NO: 14 - protein, 9 aa, Mus musculus
IIYHMDEEE

SEQ ID NO: 15 - protein, 12 aa, Mus musculus
DNYQPYPCAEDE

SEQ ID NO: 16 - protein, 9 aa, Mus musculus
DLDNYQPYP

SEQ ID NO: 17 - protein, 12 aa, Homo sapiens
GNNFDYWKYGEA

SEQ ID NO: 18 - protein, 11 aa, Homo sapiens
PDYWKYGEASS

SEQ ID NO: 19 - protein, 16 aa, Homo sapiens
ITSHDYLGQETLTEIQ

SEQ ID NO: 20 - protein, 15 aa, Mus musculus
IADHDYLGQETSTEV

SEQ ID NO: 21 - protein, 11 aa, Homo sapiens
AIAIDYDPLEG

SEQ ID NO: 22 - protein, 16 aa, Homo sapiens
PHSQYLSAEDSCPPSP

SEQ ID NO: 23 - protein, 11 aa, Mus musculus
AIAIDYDPLEG

SEQ ID NO: 24 - protein, 16 aa, Mus musculus
PHSQYLSAEDSCPPSP

SEQ ID NO: 25 - protein, 16 aa, Mus musculus
TSDVNYDSEPVPPPTP

SEQ ID NO: 26 - protein, 4 aa, Unknown
  Description of Unknown: YWTD domain peptide
YWTD

SEQ ID NO: 27 - protein, 16 aa, Artificial Sequence
  Description of Artificial Sequence: Synthetic peptide
HPELGEYPEPPPELEC

SEQ ID NO: 28 - protein, 16 aa, Artificial Sequence
  Description of Artificial Sequence: Synthetic peptide
HCRSAKANQAELENAY

SEQ ID NO: 29 - protein, 14 aa, Artificial Sequence
  Description of Artificial Sequence: Synthetic peptide
ELGEYPEPPPELEN

SEQ ID NO: 30 - protein, 188 aa, Homo sapiens
WQAFKNDATEIIPELGEYPEPPPELENNKTMNRAENGGRPPHHPFETKDVSEYSCRELHFTRYVTDGPCRSAKPVTELVCSGQCGPARLLPNAIGRGKWWRPSGPDFRCIPDRYRAQRVQLLCPGGEAPRARKVRLVASCKCKRLTRFHNQSELKDFGTEAARPQKGRKPRPRARSAKANQAELENAY

SEQ ID NO: 31 - protein, 213 aa, Homo sapiens
MQLPLALCLVCLLVHTAFRVVEGQGWQAFKNDATEIIPELGEYPEPPPELENNKTMNRAENGGRPPHHPFETKDVSEYSCRELHFTRYVTDGPCRSAKPVTELVCSGQCGPARLLPNAIGRGKWWRPSGPDFRCIPDRYRAQRVQLLCPGGEAPRARKVRLVASCKCKRLTRFHNQSELKDFGTEAARPQKGRKPRPRARSAKANQAELENAY